European Patent Application EP 4 434 350 A2, published September 25, 2024. Title: FEED ADDITIVE COMPOSITION. Applicant: International N&H Denmark ApS. The sequence listing filed with the application follows.

SEQUENCE LISTING (2 sequences)

SEQ ID NO: 1 - protein, 413 aa, Buttiauxella sp.
NDTPASGYQVEKVVILSRHGVRAPTKMTQTMRDVTPNTWPEWPVKLGYITPRGEHLISLMGGFYRQKFQQQGILSQGSCPTPNSIYVWTDVAQRTLKTGEAFLAGLAPQCGLTIHHQQNLEKADPLFHPVKAGICSMDKTQVQQAVEKEAQTPIDNLNQHYIPSLALMNTTLNFSKSPWCQKHSADKSCDLGLSMPSKLSIKDNGNEVSLDGAIGLSSTLAEIFLLEYAQGMPQAAWGNIHSEQEWALLLKLHNVYFDLMERTPYIARHKGTPLLQAISNALNPNATESKLPDISPDNKILFIAGHDTNIANIAGMLNMRWTLPGQPDNTPPGGALVFERLADKSGKQYVSVSMVYQTLEQLRSQTPLSLNQPAGSVQLKIPGCNDQTAEGYCPLSTFTRVVSQSVEPGCQLQ

SEQ ID NO: 2 - protein, 446 aa, Buttiauxella sp.
MTISAFNRKKLTLHPGLFVALSAIFSLGSTAYANDTPASGYQVEKVVILSRHGVRAPTKMTQTMRDVTPNTWPEWPVKLGYITPRGEHLISLMGGFYRQKFQQQGILSQGSCPTPNSIYVWTDVAQRTLKTGEAFLAGLAPQCGLTIHHQQNLEKADPLFHPVKAGICSMDKTQVQQAVEKEAQTPIDNLNQHYIPSLALMNTTLNFSKSPWCQKHSADKSCDLGLSMPSKLSIKDNGNEVSLDGAIGLSSTLAEIFLLEYAQGMPQAAWGNIHSEQEWALLLKLHNVYFDLMERTPYIARHKGTPLLQAISNALNPNATESKLPDISPDNKILFIAGHDTNIANIAGMLNMRWTLPGQPDNTPPGGALVFERLADKSGKQYVSVSMVYQTLEQLRSQTPLSLNQPAGSVQLKIPGCNDQTAEGYCPLSTFTRVVSQSVEPGCQLQ